European Patent Application EP 4 549 552 A1, published May 7, 2025. Title: Cardiac fibroblast cell line containing knockout of the Fhl1 gene. Applicant: Vilnius University. Application EP. The sequence listing filed with the application follows.

SEQUENCE LISTING (12 sequences)

SEQ ID NO: 1 - RNA, 24 nt, synthetic construct
  source 1..24: mol_type = other RNA
accggcttgggtacctgcggcctc

SEQ ID NO: 2 - RNA, 24 nt, synthetic construct
  source 1..24: mol_type = other RNA
aaacgaggccgcaggtacccaagc

SEQ ID NO: 3 - RNA, 24 nt, synthetic construct
  source 1..24: mol_type = other RNA
accggcacgagctgcggctccccg

SEQ ID NO: 4 - RNA, 24 nt, synthetic construct
  source 1..24: mol_type = other RNA
aaaccggggagccgcagctcgtgc

SEQ ID NO: 5 - RNA, 24 nt, synthetic construct
  source 1..24: mol_type = other RNA
accgctgctgggcttgggtacctg

SEQ ID NO: 6 - RNA, 24 nt, synthetic construct
  source 1..24: mol_type = other RNA
aaaccaggtacccaagcccagcag

SEQ ID NO: 7 - RNA, 24 nt, synthetic construct
  source 1..24: mol_type = other RNA
accgcggctccccggggacgccgg

SEQ ID NO: 8 - RNA, 24 nt, synthetic construct
  source 1..24: mol_type = other RNA
aaacccggcgtccccggggagccg

SEQ ID NO: 9 - RNA, 24 nt, synthetic construct
  source 1..24: mol_type = other RNA
accgctgctgggcttgggtacctg

SEQ ID NO: 10 - RNA, 24 nt, synthetic construct
  source 1..24: mol_type = other RNA
aaaccaggtacccaagcccagcag

SEQ ID NO: 11 - RNA, 24 nt, synthetic construct
  source 1..24: mol_type = other RNA
accggcacgagctgcggctccccg

SEQ ID NO: 12 - RNA, 23 nt, synthetic construct
  source 1..23: mol_type = other RNA
aaaccgggagccgcagctcgtgc